European Patent Application EP 4 357 366 A1, published April 24, 2024. Title: BISPECIFIC FUSION PROTEIN. Applicant: HANGZHOU SUMGEN BIOTECH CO., LTD.; SUMGEN MAB (BEIJING) BIOTECH CO., LTD. The sequence listing filed with the application follows.

SEQUENCE LISTING (28 sequences)

SEQ ID NO: 1 - protein, 104 aa, Artificial Sequence
  Ig-like domain of VEGFR1
SDTGRPFVEMYSEIPEIIHMTEGRELVIPCRVTSPNITVTLKKFPLDTLIPDGKRIIWDSRKGFIISNATYKEIGLLTCEATVNGHLYKTNYLTHRQTNTIIDV

SEQ ID NO: 2 - protein, 100 aa, Artificial Sequence
  Ig-like domain of VEGFR2
VLSPSHGIELSVGEKLVLNCTARTELNVGIDFNWEYPSSKHQHKKLVNRDLKTQSGSEMKKFLSTLTIDGVTRSDQGLYTCAASSGLMTKKNSTFVRVHE

SEQ ID NO: 3 - protein, 10 aa, Artificial Sequence
  linker
GGGGSGGGGS

SEQ ID NO: 4 - protein, 11 aa, Artificial Sequence
  LCDR1 of PD-L1 antibody 1
RASQDVSTAVA

SEQ ID NO: 5 - protein, 7 aa, Artificial Sequence
  LCDR2 of PD-L1 antibody 1
SASFLYS

SEQ ID NO: 6 - protein, 9 aa, Artificial Sequence
  LCDR3 of PD-L1 antibody 1
QQYLYHPAT

SEQ ID NO: 7 - protein, 5 aa, Artificial Sequence
  HCDR1 of PD-L1 antibody 1
DSWIH

SEQ ID NO: 8 - protein, 17 aa, Artificial Sequence
  HCDR2 of PD-L1 antibody 1
WISPYGGSTYYADSVKG

SEQ ID NO: 9 - protein, 9 aa, Artificial Sequence
  HCDR3 of PD-L1 antibody 1
RHWPGGFDY

SEQ ID NO: 10 - protein, 12 aa, Artificial Sequence
  LCDR1 of PD-L1 antibody 2
RASQRVSSSYLA

SEQ ID NO: 11 - protein, 7 aa, Artificial Sequence
  LCDR2 of PD-L1 antibody 2
DASSRAT

SEQ ID NO: 12 - protein, 9 aa, Artificial Sequence
  LCDR3 of PD-L1 antibody 2
QQYGSLPWT

SEQ ID NO: 13 - protein, 5 aa, Artificial Sequence
  HCDR1 of PD-L1 antibody 2
RYWMS

SEQ ID NO: 14 - protein, 17 aa, Artificial Sequence
  HCDR2 of PD-L1 antibody 2
NIKQDGSEKYYVDSVKG

SEQ ID NO: 15 - protein, 12 aa, Artificial Sequence
  HCDR3 of PD-L1 antibody 2
EGGWFGELAFDY

SEQ ID NO: 16 - protein, 107 aa, Artificial Sequence [sequence omitted]

SEQ ID NO: 17 - protein, 108 aa, Artificial Sequence
  light chain variable region of PD-L1 antibody 2
EIVLTQSPGTLSLSPGERATLSCRASQRVSSSYLAWYQQKPGQAPRLLIYDASSRATGIPDRFSGSGSGTDFTLTISRLEPEDFAVYYCQQYGSLPWTFGQGTKVEIK

SEQ ID NO: 18 - protein, 118 aa, Artificial Sequence [sequence omitted]

SEQ ID NO: 19 - protein, 121 aa, Artificial Sequence
  heavy chain variable region of PD-L1 antibody 2
EVQLVESGGGLVQPGGSLRLSCAASGFTFSRYWMSWVRQAPGKGLEWVANIKQDGSEKYYVDSVKGRFTISRDNAKNSLYLQMNSLRAEDTAVYYCAREGGWFGELAFDYWGQGTLVTVSS

SEQ ID NO: 20 - protein, 232 aa, Artificial Sequence
  IgG1 Fc
EPKSCDKTHTCPPCPAPELLGGPSVFLFPPKPKDTLMISRTPEVTCVVVDVSHEDPEVKFNWYVDGVEVHNAKTKPREEQYNSTYRVVSVLTVLHQDWLNGKEYKCKVSNKALPAPIEKTISKAKGQPREPQVYTLPPSRDELTKNQVSLTCLVKGFYPSDIAVEWESNGQPENNYKTTPPVLDSDGSFFLYSKLTVDKSRWQQGNVFSCSVMHEALHNHYTQKSLSLSPGK

SEQ ID NO: 21 - protein, 229 aa, Artificial Sequence
  IgG4 Fc
ESKYGPPCPPCPAPEFLGGPSVFLFPPKPKDTLMISRTPEVTCVVVDVSQEDPEVQFNWYVDGVEVHNAKTKPREEQFNSTYRVVSVLTVLHQDWLNGKEYKCKVSNKGLPSSIEKTISKAKGQPREPQVYTLPPSQEEMTKNQVSLTCLVKGFYPSDIAVEWESNGQPENNYKTTPPVLDSDGSFFLYSRLTVDKSRWQEGNVFSCSVMHEALHNHYTQKSLSLSLGK

SEQ ID NO: 22 - protein, 232 aa, Artificial Sequence
  IgG1 Fc (N298A, D357E, L359M)
EPKSCDKTHTCPPCPAPELLGGPSVFLFPPKPKDTLMISRTPEVTCVVVDVSHEDPEVKFNWYVDGVEVHNAKTKPREEQYASTYRVVSVLTVLHQDWLNGKEYKCKVSNKALPAPIEKTISKAKGQPREPQVYTLPPSREEMTKNQVSLTCLVKGFYPSDIAVEWESNGQPENNYKTTPPVLDSDGSFFLYSKLTVDKSRWQQGNVFSCSVMHEALHNHYTQKSLSLSPGK

SEQ ID NO: 23 - protein, 214 aa, Artificial Sequence
  light chain of PD-L1 antibody 1
DIQMTQSPSSLSASVGDRVTITCRASQDVSTAVAWYQQKPGKAPKLLIYSASFLYSGVPSRFSGSGSGTDFTLTISSLQPEDFATYYCQQYLYHPATFGQGTKVEIKRTVAAPSVFIFPPSDEQLKSGTASVVCLLNNFYPREAKVQWKVDNALQSGNSQESVTEQDSKDSTYSLSSTLTLSKADYEKHKVYACEVTHQGLSSPVTKSFNRGEC

SEQ ID NO: 24 - protein, 215 aa, Artificial Sequence
  light chain of PD-L1 antibody 2
EIVLTQSPGTLSLSPGERATLSCRASQRVSSSYLAWYQQKPGQAPRLLIYDASSRATGIPDRFSGSGSGTDFTLTISRLEPEDFAVYYCQQYGSLPWTFGQGTKVEIKRTVAAPSVFIFPPSDEQLKSGTASVVCLLNNFYPREAKVQWKVDNALQSGNSQESVTEQDSKDSTYSLSSTLTLSKADYEKHKVYACEVTHQGLSSPVTKSFNRGEC

SEQ ID NO: 25 - protein, 662 aa, Artificial Sequence
  heavy chain of PD-L1 antibody 1  IgG1 mutation and linker and VEGFR1R2
EVQLVESGGGLVQPGGSLRLSCAASGFTFSDSWIHWVRQAPGKGLEWVAWISPYGGSTYYADSVKGRFTISADTSKNTAYLQMNSLRAEDTAVYYCARRHWPGGFDYWGQGTLVTVSSASTKGPSVFPLAPSSKSTSGGTAALGCLVKDYFPEPVTVSWNSGALTSGVHTFPAVLQSSGLYSLSSVVTVPSSSLGTQTYICNVNHKPSNTKVDKKVEPKSCDKTHTCPPCPAPELLGGPSVFLFPPKPKDTLMISRTPEVTCVVVDVSHEDPEVKFNWYVDGVEVHNAKTKPREEQYASTYRVVSVLTVLHQDWLNGKEYKCKVSNKALPAPIEKTISKAKGQPREPQVYTLPPSREEMTKNQVSLTCLVKGFYPSDIAVEWESNGQPENNYKTTPPVLDSDGSFFLYSKLTVDKSRWQQGNVFSCSVMHEALHNHYTQKSLSLSPGKGGGGSGGGGSSDTGRPFVEMYSEIPEIIHMTEGRELVIPCRVTSPNITVTLKKFPLDTLIPDGKRIIWDSRKGFIISNATYKEIGLLTCEATVNGHLYKTNYLTHRQTNTIIDVVLSPSHGIELSVGEKLVLNCTARTELNVGIDFNWEYPSSKHQHKKLVNRDLKTQSGSEMKKFLSTLTIDGVTRSDQGLYTCAASSGLMTKKNSTFVRVHE

SEQ ID NO: 26 - protein, 665 aa, Artificial Sequence
  heavy chain of PD-L1 antibody 2  IgG1 and linker and VEGFR1R2
EVQLVESGGGLVQPGGSLRLSCAASGFTFSRYWMSWVRQAPGKGLEWVANIKQDGSEKYYVDSVKGRFTISRDNAKNSLYLQMNSLRAEDTAVYYCAREGGWFGELAFDYWGQGTLVTVSSASTKGPSVFPLAPSSKSTSGGTAALGCLVKDYFPEPVTVSWNSGALTSGVHTFPAVLQSSGLYSLSSVVTVPSSSLGTQTYICNVNHKPSNTKVDKRVEPKSCDKTHTCPPCPAPEFEGGPSVFLFPPKPKDTLMISRTPEVTCVVVDVSHEDPEVKFNWYVDGVEVHNAKTKPREEQYNSTYRVVSVLTVLHQDWLNGKEYKCKVSNKALPASIEKTISKAKGQPREPQVYTLPPSREEMTKNQVSLTCLVKGFYPSDIAVEWESNGQPENNYKTTPPVLDSDGSFFLYSKLTVDKSRWQQGNVFSCSVMHEALHNHYTQKSLSLSPGKGGGGSGGGGSSDTGRPFVEMYSEIPEIIHMTEGRELVIPCRVTSPNITVTLKKFPLDTLIPDGKRIIWDSRKGFIISNATYKEIGLLTCEATVNGHLYKTNYLTHRQTNTIIDVVLSPSHGIELSVGEKLVLNCTARTELNVGIDFNWEYPSSKHQHKKLVNRDLKTQSGSEMKKFLSTLTIDGVTRSDQGLYTCAASSGLMTKKNSTFVRVHE

SEQ ID NO: 27 - protein, 659 aa, Artificial Sequence
  heavy chain of PD-L1 of antibody 1  IgG4 and linker and VEGFR1R2
EVQLVESGGGLVQPGGSLRLSCAASGFTFSDSWIHWVRQAPGKGLEWVAWISPYGGSTYYADSVKGRFTISADTSKNTAYLQMNSLRAEDTAVYYCARRHWPGGFDYWGQGTLVTVSSASTKGPSVFPLAPCSRSTSESTAALGCLVKDYFPEPVTVSWNSGALTSGVHTFPAVLQSSGLYSLSSVVTVPSSSLGTKTYTCNVDHKPSNTKVDKRVESKYGPPCPPCPAPEFLGGPSVFLFPPKPKDTLMISRTPEVTCVVVDVSQEDPEVQFNWYVDGVEVHNAKTKPREEQFNSTYRVVSVLTVLHQDWLNGKEYKCKVSNKGLPSSIEKTISKAKGQPREPQVYTLPPSQEEMTKNQVSLTCLVKGFYPSDIAVEWESNGQPENNYKTTPPVLDSDGSFFLYSRLTVDKSRWQEGNVFSCSVMHEALHNHYTQKSLSLSLGKGGGGSGGGGSSDTGRPFVEMYSEIPEIIHMTEGRELVIPCRVTSPNITVTLKKFPLDTLIPDGKRIIWDSRKGFIISNATYKEIGLLTCEATVNGHLYKTNYLTHRQTNTIIDVVLSPSHGIELSVGEKLVLNCTARTELNVGIDFNWEYPSSKHQHKKLVNRDLKTQSGSEMKKFLSTLTIDGVTRSDQGLYTCAASSGLMTKKNSTFVRVHE

SEQ ID NO: 28 - protein, 204 aa, Artificial Sequence
  Ig-like domain of VEGFR1 and Ig-like domain of VEGFR2
SDTGRPFVEMYSEIPEIIHMTEGRELVIPCRVTSPNITVTLKKFPLDTLIPDGKRIIWDSRKGFIISNATYKEIGLLTCEATVNGHLYKTNYLTHRQTNTIIDVVLSPSHGIELSVGEKLVLNCTARTELNVGIDFNWEYPSSKHQHKKLVNRDLKTQSGSEMKKFLSTLTIDGVTRSDQGLYTCAASSGLMTKKNSTFVRVHE